European Patent Application EP 4 549 559 A1, published May 7, 2025. Title: 一种提高植酸酶热稳定性的方法及突变体和应用. Applicant: Beijing Institute of Animal Husbandry and Veterinary Medicine of Chinese Academy of Agricultural Sciences. The sequence listing filed with the application follows.

SEQUENCE LISTING (33 sequences)

SEQ ID NO: 1 - protein, 418 aa, synthetic construct
AAPVAIQPTGYTLERVVILSRHGVRSPTKQTQLMNDVTPDTWPQWPVAAGELTPRGAQLVTLMGGFYGDYFRSQGLLAAGCPTDADIYAQADVDQRTRLTGQAFLDGIAPGCGLKVHYQADLKKVDPLFHPVDAGVCKLDSTQTHKAVEERLGGPLSELSKRYAKPFAQMGEILNFAASPYCKSLQQQGKTCDFANFAANKITVNKPGTKVSLSGPLALSSTLGEIFLLQNSQAMPDVAWHRLTGEDNWISLLSLHNAQFDLMAKTPYIARHKGTPLLQQIETALVLQRDAQGQTLPLSPQTKILFLGGHDTNIANIAGMLGLNWQLPQQPDNTPPGGGLVFELWQNPDNHQRYVAVKLFYQTMGQLRNAEKLDLKNNPAGRVPVAIDGCENSGDDKLCQLDTFQKKVAQAIEPACHI

SEQ ID NO: 2 - protein, 418 aa, synthetic construct
AAPVAIQPTGYTLERVVILSRHGVRSPTKQTQLMNDVTPDTWPQWPVAAGELTPRGCQLVTLMGGFYGDYFRSQGLLAAGCPTDADIYAQADVDQRTRLTCQCFLDGIAPGCGLKCHYQADLKKVDPLFHPVDAGVCKLDSTQTHKCVEERLGGPLSELSKRYAKPFAQMGEILNFAASPYCKSLQQQGKTCDFANFAANKITVNKPGTKVSLSGPLALSSTLGEIFLLQNSQAMPDVAWHRLTGEDNWISLLSLHNAQFDLMAKTPCIACHKGTPLLQQIETALVLQRDAQGQTLPLSPQTKILFLGGHDTNIANIAGMLGLNWQLPQQPDNTPPGGGLVFELWQNPDNHQCYVAVKLFYQTMGQLRNAEKLDLKNNPAGRVPVAIDGCENSGDDKLCQCDTFQKKVAQAICPACHI

SEQ ID NO: 3 - protein, 418 aa, synthetic construct
AAPVAIQPTGYTLERVVILSRHGVRSPTKQTQLMNDVTPDTWPQWPVAAGELTPRGCQLVTLMGRFYGDYFRSQGLLAAGCPTDADIYAQADVDQRTRLTCQCFLDGIAPGCGLKCHYQADLKKVDPLFHPVDAGVCKLDSTQTHKCVEERLGGPLSELSKRYAKPFAQMGEILNFAASPYCKSLQQQGKTCDFANFAANKITVNKPGTKVSLSGPLALSSTLGEIFLLQNSQAMPDVAWHRLTGEDNWISLLSLHNAQFDLMAKTPCIACHKGTPLLQQILTALVLQRDAQGQTLPLSPQTKILFLGGHDTNIANIAGMLGLNWQLPQQPDNTPPGGGLVFELWQNPDNHQCYVAVKLFYQTMDQLRNAEKLDLKNNPAGRVPVAIDGCENSGDDKLCQCDTFQKKVAQAICPACHI

SEQ ID NO: 4 - protein, 418 aa, synthetic construct
AAPVAIQPTGYTLERVVILSRHGVRSPTKQTQLMNDVTPDTWPQWPVAAGELTPRGCQLVTLMGRFYGDYFRSQGLLAAGCPTDADIYAQADVDQRTRLTCQCFLDGIAPGCGLKCHYQADLKKVDPLFHPVEAGVCKLDSTQTHKCVEERLGGPLSELSKRYAKPFAQMGEILNFAASPYCKSLQQQGKTCDFANFAANKITVNKPGTKVSLSGPLALSSTLGEIFLLQNSQAMPDVAWHRLTGEDNWISLLSLHNAQFDLMAKTPCIACHKGTPLLQQILTALVLQRDAQGQTLPLSPQTKILFLGGHDTNIANIAGMLGLNWQLPQQPDNTPPGGGLVFELWQNPDNHQCYVAVKLFYQTMDQLRNAEKLDLKNNPAGIVPVAIDGCENIGDDKLCQCDTFQKKVAQAICPACHI

SEQ ID NO: 5 - DNA, 1258 bp, synthetic construct
  source 1..1258: mol_type = other DNA
gctgctccagtcgctatccaacctactggttacactcttgagagagttgtcatcttgtctagacatggtgttagatccccaactaagcagacccaattgatgaacgatgtgacacctgacacgtggcctcaatggccagttgcagctggtgagttgacaccaagaggttgtcagttggttactttgatgggtggattctacggtgactatttcagatcccaaggattgcttgctgccggctgtcctactgatgctgacatctacgcacaagctgacgttgatcaaagaactcgtttgacctgtcaatgtttcttggatggtatcgctccaggatgtggcttgaaatgtcactaccaggctgatttgaagaaggttgatccactgttccaccctgttgatgcaggtgtttgtaagcttgactctactcaaacccacaaatgtgttgaagagagattgggtggtccattgagcgaactttcgaagagatacgccaaaccttttgcacaaatgggagagatcctgaacttcgcagcgtcaccttactgtaagagtttgcaacagcaaggtaagacttgcgactttgccaacttcgctgccaacaagatcactgtcaacaagcctggaacgaaagtatccttgtctggtccattggctctgtcttccactcttggagaaatcttcttgctgcaaaactctcaagctatgccagatgttgcctggcacagattgaccggtgaggacaactggatttctttgctctccttacacaatgcccaattcgatctgatggcaaagactccttgtattgcttgtcacaaaggaactcccttgcttcagcaaatcgaaactgctttggtcctccaaagggacgcccagggtcaaactttgccattgtctcctcagaccaagatcctgttcttgggtggacacgatactaacatcgcaaacatcgctgggatgttgggtttgaactggcaacttccacagcaaccagacaacaccccacctggcggtggtctagtcttcgagttgtggcaaaaccctgacaaccaccagtgttacgttgctgtaaagttgttctatcagactatgggacaattgcgtaacgcagagaagttggatttgaagaacaacccagccggtagggttcctgtcgcaattgacggttgtgagaactctggagatgacaagttgtgccagtgtgatactttccagaagaaggttgctcaggccatattgtccagcttgtcacatctaa

SEQ ID NO: 6 - DNA, 1258 bp, synthetic construct
  source 1..1258: mol_type = other DNA
gctgctccagtcgctatccaacctactggttacactcttgagagagttgtcatcttgtctagacatggtgttagatccccaactaagcagacccaattgatgaacgatgtgacacctgacacgtggcctcaatggccagttgcagctggtgagttgacaccaagaggttgtcagttggttactttgatgggtagattctacggtgactatttcagatcccaaggattgcttgctgccggctgtcctactgatgctgacatctacgcacaagctgacgttgatcaaagaactcgtttgacctgtcaatgtttcttggatggtatcgctccaggatgtggcttgaaatgtcactaccaggctgatttgaagaaggttgatccactgttccaccctgttgatgcaggtgtttgtaagcttgactctactcaaacccacaaatgtgttgaagagagattgggtggtccattgagcgaactttcgaagagatacgccaaaccttttgcacaaatgggagagatcctgaacttcgcagcgtcaccttactgtaagagtttgcaacagcaaggtaagacttgcgactttgccaacttcgctgccaacaagatcactgtcaacaagcctggaacgaaagtatccttgtctggtccattggctctgtcttccactcttggagaaatcttcttgctgcaaaactctcaagctatgccagatgttgcctggcacagattgaccggtgaggacaactggatttctttgctctccttacacaatgcccaattcgatctgatggcaaagactccttgtattgcttgtcacaaaggaactcccttgcttcagcaaatcttgactgctttggtcctccaaagggacgcccagggtcaaactttgccattgtctcctcagaccaagatcctgttcttgggtggacacgatactaacatcgcaaacatcgctgggatgttgggtttgaactggcaacttccacagcaaccagacaacaccccacctggcggtggtctagtcttcgagttgtggcaaaaccctgacaaccaccagtgttacgttgctgtaaagttgttctatcagactatggatcaattgcgtaacgcagagaagttggatttgaagaacaacccagccggtagggttcctgtcgcaattgacggttgtgagaactctggagatgacaagttgtgccagtgtgatactttccagaagaaggttgctcaggccatattgtccagcttgtcacatctaa

SEQ ID NO: 7 - DNA, 1258 bp, synthetic construct
  source 1..1258: mol_type = other DNA
gctgctccagtcgctatccaacctactggttacactcttgagagagttgtcatcttgtctagacatggtgttagatccccaactaagcagacccaattgatgaacgatgtgacacctgacacgtggcctcaatggccagttgcagctggtgagttgacaccaagaggttgtcagttggttactttgatgggtagattctacggtgactatttcagatcccaaggattgcttgctgccggctgtcctactgatgctgacatctacgcacaagctgacgttgatcaaagaactcgtttgacctgtcaatgtttcttggatggtatcgctccaggatgtggcttgaaatgtcactaccaggctgatttgaagaaggttgatccactgttccaccctgttgaagcaggtgtttgtaagcttgactctactcaaacccacaaatgtgttgaagagagattgggtggtccattgagcgaactttcgaagagatacgccaaaccttttgcacaaatgggagagatcctgaacttcgcagcgtcaccttactgtaagagtttgcaacagcaaggtaagacttgcgactttgccaacttcgctgccaacaagatcactgtcaacaagcctggaacgaaagtatccttgtctggtccattggctctgtcttccactcttggagaaatcttcttgctgcaaaactctcaagctatgccagatgttgcctggcacagattgaccggtgaggacaactggatttctttgctctccttacacaatgcccaattcgatctgatggcaaagactccttgtattgcttgtcacaaaggaactcccttgcttcagcaaatcttgactgctttggtcctccaaagggacgcccagggtcaaactttgccattgtctcctcagaccaagatcctgttcttgggtggacacgatactaacatcgcaaacatcgctgggatgttgggtttgaactggcaacttccacagcaaccagacaacaccccacctggcggtggtctagtcttcgagttgtggcaaaaccctgacaaccaccagtgttacgttgctgtaaagttgttctatcagactatggatcaattgcgtaacgcagagaagttggatttgaagaacaacccagccggtattgttcctgtcgcaattgacggttgtgagaacattggagatgacaagttgtgccagtgtgatactttccagaagaaggttgctcaggccatattgtccagcttgtcacatctaa

SEQ ID NO: 8 - DNA, 23 bp, synthetic construct
  source 1..23: mol_type = other DNA
acccacaaatgtgttgaagagag

SEQ ID NO: 9 - DNA, 23 bp, synthetic construct
  source 1..23: mol_type = other DNA
tctagcaatacaaggagtctttg

SEQ ID NO: 10 - DNA, 25 bp, synthetic construct
  source 1..25: mol_type = other DNA
tacattgcttgtcacaaaggaactc

SEQ ID NO: 11 - DNA, 28 bp, synthetic construct
  source 1..28: mol_type = other DNA
acaagctggacatatggcctgagcaacc

SEQ ID NO: 12 - DNA, 47 bp, synthetic construct
  source 1..47: mol_type = other DNA
tcctggagcgataccatccaagaatgcttgacaggtcaaacgagttc

SEQ ID NO: 13 - DNA, 49 bp, synthetic construct
  source 1..49: mol_type = other DNA
ttcttggatggtatcgctccaggatgtggcttgaaatgtcactaccagg

SEQ ID NO: 14 - DNA, 25 bp, synthetic construct
  source 1..25: mol_type = other DNA
caccaagaggttgtcagttggttac

SEQ ID NO: 15 - DNA, 27 bp, synthetic construct
  source 1..27: mol_type = other DNA
catccaagaaacattgtccggtcaaac

SEQ ID NO: 16 - DNA, 28 bp, synthetic construct
  source 1..28: mol_type = other DNA
caaccaccagtgttacgttgctgtaaag

SEQ ID NO: 17 - DNA, 22 bp, synthetic construct
  source 1..22: mol_type = other DNA
gaaagtatcacactggcacaac

SEQ ID NO: 18 - DNA, 34 bp, synthetic construct
  source 1..34: mol_type = other DNA
agcaacgtaacactggtggttgtcagggttttgc

SEQ ID NO: 19 - DNA, 27 bp, synthetic construct
  source 1..27: mol_type = other DNA
gccagtgtgatactttccagaagaagg

SEQ ID NO: 20 - DNA, 30 bp, synthetic construct
  source 1..30: mol_type = other DNA
cagactatggatcaattgcgtaacgcagag

SEQ ID NO: 21 - DNA, 30 bp, synthetic construct
  source 1..30: mol_type = other DNA
cgcaattgatccatagtctgatagaacaac

SEQ ID NO: 22 - DNA, 32 bp, synthetic construct
  source 1..32: mol_type = other DNA
gacatctacgttcaagctgacgttgatcaaag

SEQ ID NO: 23 - DNA, 32 bp, synthetic construct
  source 1..32: mol_type = other DNA
gtcagcttgaacgtagatgtcagcatcagtag

SEQ ID NO: 24 - DNA, 29 bp, synthetic construct
  source 1..29: mol_type = other DNA
atgggtagattctacggtgactatttcag

SEQ ID NO: 25 - DNA, 31 bp, synthetic construct
  source 1..31: mol_type = other DNA
accgtagaatctacccatcaaagtaaccaac

SEQ ID NO: 26 - DNA, 32 bp, synthetic construct
  source 1..32: mol_type = other DNA
cagcaaatcttgactgctttggtcctccaaag

SEQ ID NO: 27 - DNA, 32 bp, synthetic construct
  source 1..32: mol_type = other DNA
caaagcagtcaagatttgctgaagcaagggag

SEQ ID NO: 28 - DNA, 31 bp, synthetic construct
  source 1..31: mol_type = other DNA
caccctgttgaagcaggtgtttgtaagcttg

SEQ ID NO: 29 - DNA, 31 bp, synthetic construct
  source 1..31: mol_type = other DNA
aaacacctgcttcaacagggtggaacagtgg

SEQ ID NO: 30 - DNA, 31 bp, synthetic construct
  source 1..31: mol_type = other DNA
ccagccggtattgttcctgtcgcaattgacg

SEQ ID NO: 31 - DNA, 31 bp, synthetic construct
  source 1..31: mol_type = other DNA
gacaggaacaataccggctgggttgttcttc

SEQ ID NO: 32 - DNA, 31 bp, synthetic construct
  source 1..31: mol_type = other DNA
tgtgagaacattggagatgacaagttgtgcc

SEQ ID NO: 33 - DNA, 32 bp, synthetic construct
  source 1..32: mol_type = other DNA
gtcatctccaatgttctcacaaccgtcaattg